European Patent Specification EP 3 596 110 B1, published September 4, 2024. Title: Bordetella vaccines comprising LPS with reduced reactogenicity. Applicant: De Staat der Nederlanden, vert. door de minister van VWS, Ministerie van Volksgezondheid, Welzijn en Sport. The sequence listing filed with the application follows.

SEQUENCE LISTING (32 sequences)

SEQ ID NO: 1 - protein, 258 aa, Pseudomonas aeruginosa
MSLIDPRAIIDPSARLAADVQVGPWSIVGAEVEIGEGTVIGPHVVLKGPTKIGKHNRIYQFSSVGEDTPDLKYKGEPTRLVIGDHNVIREGVTIHRGTVQDRAETTIGDHNLIMAYAHIGHDSVIGNHCILVNNTALAGHVHVDDWAILSGYTLVHQYCRIGAHSFSGMGSAIGKDVPAYVTVFGNPAEARSMNFEGMRRRGFSSEAIHALRRAYKVVYRQGHTVEEALAELAESAAQFPEVAVFRDSIQSATRGITR

SEQ ID NO: 2 - protein, 289 aa, Neisseria meningitidis
MKFIFFVLYVLQFLPFALLHKIADLTGLLAYLLVKPRRRIGEINLAKCFSEWSEEKRKTVLKQHFKHMAKLMLEYGLYWYAPAGRLKSLVRYRNKHYLDDALAAGEKVIILYPHFTAFEMAVYALNQDIPLISMYSHQKNKILDEQILKGRNRYHNVFLIGRTEGLRALVKQFRKSSAPFLYLPDQDFGRNDSVFVDFFGIQTATITGLSRIAALANAKVIPAIPVREADNTVTLHFYPAWKSFPGEDAKADAQRMNRFIEDRVREHPEQYFWLHKRFKTRPEGSPDFY

SEQ ID NO: 3 - protein, 288 aa, Porphyromonas gingivalis
MQAVLPLWMVRLQSRILAGLLHTVVRYRRKVVRDNLTRCFPEKSLQEIRRIERRFYYNFTYQILSSFKLLTYSQTQLRRHISFENLDVLIRLRAEGHPAILLMMGHFGNWEYFSGSQAIIKDLGLQIYQIFRPLKSTSSDRLMHRIRERFGSRGIAKHDVPRELLRLVRNPIPTETPLVIFIADQSPAYAGSYWTTFFGRETAFFNGTEKLGHKFSLPVVYMDVEKTGHDVFTGTIKLLHHPQDDSPEGSITEEYVRLMEATIRRDPSQWLWSHRRWKRPRLHNTRQP

SEQ ID NO: 4 - protein, 353 aa, Pseudomonas aeruginosa
MMSTLSYTLGQLAAHVGAEVRGDADLPIQGLATLQEAGPAQLSFLANPQYRKYLPESRAGAVLLTAADADGFAGTALVVANPYLAYASLSHLFDRKPKAAAGIHPTAIVAADAEVDPSASVGAYAVIESGARIGAGVSIGAHCVIGARSVIGEGGWLAPRVTLYHDVTIGARVSIQSGAVIGGEGFGFANEKGVWQKIAQIGGVTIGDDVEIGANTTIDRGALSDTLIGNGVKLDNQIMIAHNVQIGDHTAMAACVGISGSAKIGRHCMLAGGVGLVGHIEICDNVFVTGMTMVTRSITEPGSYSSGTAMQPAAEWKKSAARIRQLDDMARRLQQLEKRLAAVTSSGDASSDA

SEQ ID NO: 5 - protein, 240 aa, Neisseria meningitidis
MKPAYFISDLHLSEKQPELTALLLRFLRSSAARQARAVYILGDLFDFWVGDDEVSELNTSVAREIRKLSDKGVAVFFVRGNRDFLIGQNFCRQAGMTLLPDYSVLDLFGCKTLICHGDTLCTDDRAYQRFRKIVHRKRLQKLFLMLPLKWRTRLATKIRRVSKMEKQVKPADIMDVNAAFTARQVRAFGAERLIHGHTHREHIHHENGFTRIVLGDWHNDYASILRVDGDGAVFVPLEKY

SEQ ID NO: 6 - protein, 258 aa, Neisseria meningitidis
MTLIHPTAVIDPKAELDSGVKVGAYTVIGPNVQIGANTEIGPHAVINGHTSIGENNRIFQFASLGEIPQDKKYRDEPTKLIIGNGNTIREFTTFNLGTVTGIGETRIGDDNWIMAYCHLAHDCVIGNHTIFANNASLAGHVTIGDYVVLGGYTLVFQFCRIGDYAMTAFAAGVHKDVPPYFMASGYRAEPAGLNSEGMRRNGFTAEQISAVKDVYKTLYHRGIPFEEAKADILRRAETQAELAVFRDFFAQSARGIIR

SEQ ID NO: 7 - DNA, 33 bp, artificial
  primer
aagcgcgccatatgaccctcatccacccgaccg

SEQ ID NO: 8 - DNA, 41 bp, artificial
  primer
aagcgcgcaagctttcagcggatgatgccgcgtgccgattg

SEQ ID NO: 9 - DNA, 31 bp, artificial
  primer
aagcgcgccatatgagtttgatcgatcctcg

SEQ ID NO: 10 - DNA, 41 bp, artificial
  primer
aagcgcgaagcttatcagcgggtgatgccgcgggttgcgct

SEQ ID NO: 11 - DNA, 34 bp, artificial
  primer
aacgcgcgcatatgaaatttatattttttgtact

SEQ ID NO: 12 - DNA, 40 bp, artificial
  primer
aagcgcgcaagctttcagtaaaaatcggggctgccttccg

SEQ ID NO: 13 - DNA, 31 bp, artificial
  primer
aagcgcgccatatgaaagcgacactttccct

SEQ ID NO: 14 - DNA, 37 bp, artificial
  primer
aagcgcgcaagctttcatagttgtcgggtattatgca

SEQ ID NO: 15 - DNA, 20 bp, artificial
  primer
gtccaaatcggcgcgaatac

SEQ ID NO: 16 - DNA, 20 bp, artificial
  primer
ctttgacggcggaaatctgc

SEQ ID NO: 17 - DNA, 20 bp, artificial
  primer
ccattggcgaccacaacctg

SEQ ID NO: 18 - DNA, 20 bp, artificial
  primer
tgccgaagaccgtcacgtag

SEQ ID NO: 19 - DNA, 20 bp, artificial
  primer
tgaaatcgctggtgcgctac

SEQ ID NO: 20 - DNA, 20 bp, artificial
  primer
atcgggcagatacagaaacg

SEQ ID NO: 21 - DNA, 20 bp, artificial
  primer
gtgctaccgctatggatggt

SEQ ID NO: 22 - DNA, 20 bp, artificial
  primer
ctataccacgcgaaccgaat

SEQ ID NO: 23 - DNA, 20 bp, artificial
  primer
ctatgtggcgcggtattatc

SEQ ID NO: 24 - DNA, 20 bp, artificial
  primer
caactttatccgcctccatc

SEQ ID NO: 25 - protein, 178 aa, Bordetella parapertussis
MQFLKKNKPLFGIVTLALACATAQAQPTQGGVSLHYGIGDHYQRVTLNYETPTLWSHQFGGNWGRLDLTPELGASYWWADGSRSPGHVWQASAIPMFRWWTGERFYIEAGIGATVFSSTSFADKRIGSAFQFGDHIGLGFLLTPSNRIGLRYSHFSNAGIKEPNPGLDIVQLTYTYQF

SEQ ID NO: 26 - DNA, 29 bp, artificial
  primer
cgcgcgcatatgatgagtaccttgtccta

SEQ ID NO: 27 - DNA, 60 bp, artificial
  primer
gcgcgcaagcttttaatgatgatgatgatgatgatgatggccgccgcccgcatcagatga

SEQ ID NO: 28 - protein, 264 aa, Bordetella pertussis
MSGNIHPTAVVDPAAQIDSSVVIGPYSVVGPGVSIAAGTEVGAHCVLDGVTSIGRDNRFYRFCSIGGMPQDKKYSGEPTRLVIGDRNTVREFTTFNTGTVQDGGVTSIGDDNWIMAYVHIAHDCHIGNNTILANSVQLGGHVQVGDWAIVGGLTGVHQFAKIGAHSMTGGNSSLMQDAPPFVLAAGNPCRPVGVNVEGLKRRGFSAAAISALRDAYKSIYRRGLSLDEGRAELRARQQAEPDVAEHLQTMLDFLDASTRGIIRP

SEQ ID NO: 29 - protein, 363 aa, Bordetella pertussis
MPVLLDPENALALDVLLAGIDAQGLDWHLSAPDAADLPRIRGIGTLSSAGNEEISFLSNPRYQNQLATTRAAAVIVTPDVAQARQEQGASGHVLVVCKHPYLLYARLAQWFERASRPAGPAGVHPSAVVDPSAEIDADVRVGAQCVIEAGARIGRGARLGPGCVIGAGSTVGADSLLHPRVTLYAGVHVGERAIIHSGAVLGADGFGFAPDPTLGRGAWGKIPQLGEVRVGNDVEIGANTTIDRGALDDTIVGDGVKLDNQIMVAHNVRIGAHTAIAACVGIAGSTTIGERCTIGGASMLSGHLAIADDVNISGGTAVTSNIAKAGRYTGVYPYAEHSEWQRNAAVIQQLALLRRRLRALERE

SEQ ID NO: 30 - protein, 249 aa, Bordetella pertussis
MWLASDLHLGPATPATAEAFLGLLQAAADEASALLLPGDIFDAWIGDDVIRAAPPWLAAVLHGIRAAAGRIPVYLGRGNRDFLIGQELADALGAHLLPEPVLLETDYGRILLTHGDEYCTDDSAYQQFRAMVRNPQWQAQFLAKSIPERLAMAEQARGESQAANQAKSMEIMDVNPAAVEAALREADVDVLVHGHTHRPARHVLSVDGRKRERWVLPDWDCDHADPPRGGWLVIDRDGLQCFDLVEDED

SEQ ID NO: 31 - protein, 296 aa, Bordetella pertussis
MSQFKTRALTAMLRGFARMRPATRQRAGALVGWLSYRLARSRVRIVRRNLELCFPGQPEAVRERWTREHFRALGQSIVDRGVLWYGSPEAVREMVTQTGAERINALIAAGRPVILLAPHFVALDAAATRLTMEVPSGATMYTPQSDPAVDAIVRAGRARFNEVFLVSRKDGVRDLVRHLREPRPVYYLPDMDFGRAGSIFVPFFGVPAATLLATAQLARKWNAAVLPILDFWDPRTGRYHVEVLPELPDFPGDGSLEDATTRLNRELESWVLRCPSQYYWVHRRFKTRPLGKPKLY

SEQ ID NO: 32 - protein, 468 aa, Pseudomonas aeruginosa
MSAWRHLSLWMNQLDDPLEARPSLEESLEVDVAIVGAGYTGLWTAYYLKRRAPQLRVAIVEAETAGFGASGRNGGWLMGNLLGEDGLLAGLPPERRRAGYDLLHGIPDEVARVLQEEGIDCDYRKGGVLYCAARYPEQERRLRAYLHDLYAEGLDESDYRWLTPQELDQQLRIPGSYGAIHSPHCATIQPARLARGLARAVERLGVRLFEKSRVLHWQRGLLRTERGELRAEWIVPAVEGYAASLPPLGHYQLPVQSLLVATEPLPSSVWAEIGLERGQAFSEFSRQVTYGQRTADDRLAFGARGGYRFGGKLRSDFSLDDEEVGLRRYLFGELFPLLKDARISHTWGGNLGMARRFRPHMLLDRASGIALSGGYGGEGVGASNLGGRTLAALILGEDSELLRQPWVLGERPLDSLARWEPEPCRWLGYNAIIRSFVHEDRVLADPHSAPWRRSLAQTLAAGMESLMR